European Patent Application EP 4 703 472 A1, published March 4, 2026. Title: Non-naturally occurring polynucleotide for alteration of target nucleotide sequence. Applicant: Ｅｕｒｕｓ　Ｔｈｅｒａｐｅｕｔｉｃｓ株式会社. The sequence listing filed with the application follows.

SEQUENCE LISTING (240 sequences)

SEQ ID NO: 1 - DNA, 534 bp, Oplophorus gracilirostris
  source 1..534: mol_type = genomic DNA
ggtaaagccaccatggtcttcacactcgaagatttcgttggggactggcgacagacagccggctacaacctggaccaagtccttgaacagggaggtgtgtccagtttgtttcagaatctcggggtgtccgtaactccgatccaaaggattgtcctgagcggtgaaaatgggctgaagatcgacatccatgtcatcatcccgtatgaaggtctgagcggcgaccaaatgggccagatcgaaaaaatttttaaggtggtgtaccctgtggatgatcatcactttaaggtgatcctgcactatggcacactggtaatcgacggggttacgccgaacatgatcgactatttcggacggccgtatgaaggcatcgccgtgttcgacggcaaaaagatcactgtaacagggaccctgtggaacggcaacaaaattatcgacgagcgcctgatcaaccccgacggctccctgctgttccgagtaaccatcaacggagtgaccggctggcggctgtgcgaacgcattctggcgtaattctag

SEQ ID NO: 2 - DNA, 21 bp, synthetic construct
  source 1..21: mol_type = other DNA
  misc_feature 11: note = LNA
tcaaggacttggtccaggttg

SEQ ID NO: 3 - DNA, 21 bp, synthetic construct
  source 1..21: mol_type = other DNA
  misc_feature 10: note = LNA
  misc_feature 12: note = LNA
tcaaggacttggtccaggttg

SEQ ID NO: 4 - DNA, 21 bp, synthetic construct
  source 1..21: mol_type = other DNA
  misc_feature 1: note = LNA
  misc_feature 11: note = LNA
tcaaggacttggtccaggttg

SEQ ID NO: 5 - DNA, 21 bp, synthetic construct
  source 1..21: mol_type = other DNA
  misc_feature 1: note = LNA
  misc_feature 10: note = LNA
  misc_feature 12: note = LNA
tcaaggacttggtccaggttg

SEQ ID NO: 6 - DNA, 25 bp, synthetic construct
  source 1..25: mol_type = other DNA
  misc_feature 13: note = LNA
gttcaaggacttggtccaggttgta

SEQ ID NO: 7 - DNA, 25 bp, synthetic construct
  source 1..25: mol_type = other DNA
  misc_feature 12: note = LNA
  misc_feature 14: note = LNA
gttcaaggacttggtccaggttgta

SEQ ID NO: 8 - DNA, 25 bp, synthetic construct
  source 1..25: mol_type = other DNA
  misc_feature 1: note = LNA
  misc_feature 13: note = LNA
gttcaaggacttggtccaggttgta

SEQ ID NO: 9 - DNA, 25 bp, synthetic construct
  source 1..25: mol_type = other DNA
  misc_feature 1: note = LNA
  misc_feature 12: note = LNA
  misc_feature 14: note = LNA
gttcaaggacttggtccaggttgta

SEQ ID NO: 10 - DNA, 25 bp, synthetic construct
  source 1..25: mol_type = other DNA
  misc_feature 1: note = LNA
gttcaaggacttggtccaggttgta

SEQ ID NO: 11 - DNA, 25 bp, synthetic construct
  source 1..25: mol_type = other DNA
  misc_feature 25: note = LNA
gttcaaggacttggtccaggttgta

SEQ ID NO: 12 - DNA, 25 bp, synthetic construct
  source 1..25: mol_type = other DNA
gttcaaggacttggtccaggttgta

SEQ ID NO: 13 - DNA, 25 bp, synthetic construct
  source 1..25: mol_type = other DNA
  misc_feature 1: note = LNA
  misc_feature 12: note = LNA
  misc_feature 14: note = LNA
gttcaaggacttagtccaggttgta

SEQ ID NO: 14 - DNA, 29 bp, synthetic construct
  source 1..29: mol_type = other DNA
  misc_feature 1: note = LNA
  misc_feature 14: note = LNA
  misc_feature 16: note = LNA
ctgttcaaggacttggtccaggttgtagc

SEQ ID NO: 15 - DNA, 31 bp, synthetic construct
  source 1..31: mol_type = other DNA
  misc_feature 1: note = LNA
  misc_feature 15: note = LNA
  misc_feature 17: note = LNA
cctgttcaaggacttggtccaggttgtagcc

SEQ ID NO: 16 - DNA, 35 bp, synthetic construct
  source 1..35: mol_type = other DNA
  misc_feature 1: note = LNA
  misc_feature 17: note = LNA
  misc_feature 19: note = LNA
tccctgttcaaggacttggtccaggttgtagccgg

SEQ ID NO: 17 - DNA, 41 bp, synthetic construct
  source 1..41: mol_type = other DNA
  misc_feature 1: note = LNA
  misc_feature 20: note = LNA
  misc_feature 22: note = LNA
acctccctgttcaaggacttggtccaggttgtagccggctg

SEQ ID NO: 18 - DNA, 45 bp, synthetic construct
  source 1..45: mol_type = other DNA
  misc_feature 1: note = LNA
  misc_feature 22: note = LNA
  misc_feature 24: note = LNA
acacctccctgttcaaggacttggtccaggttgtagccggctgtc

SEQ ID NO: 19 - DNA, 49 bp, synthetic construct
  source 1..49: mol_type = other DNA
  misc_feature 1: note = LNA
  misc_feature 24: note = LNA
  misc_feature 26: note = LNA
acacacctccctgttcaaggacttggtccaggttgtagccggctgtctg

SEQ ID NO: 20 - DNA, 53 bp, synthetic construct
  source 1..53: mol_type = other DNA
  misc_feature 1: note = LNA
  misc_feature 26: note = LNA
  misc_feature 28: note = LNA
ggacacacctccctgttcaaggacttggtccaggttgtagccggctgtctgtc

SEQ ID NO: 21 - DNA, 75 bp, synthetic construct
  source 1..75: mol_type = other DNA
  misc_feature 1: note = LNA
  misc_feature 37: note = LNA
  misc_feature 39: note = LNA
tgaaacaaactggacacacctccctgttcaaggacttggtccaggttgtagccggctgtctgtcgccagtcccca

SEQ ID NO: 22 - DNA, 95 bp, synthetic construct
  source 1..95: mol_type = other DNA
  misc_feature 1: note = LNA
  misc_feature 47: note = LNA
  misc_feature 49: note = LNA
cccgagattctgaaacaaactggacacacctccctgttcaaggacttggtccaggttgtagccggctgtctgtcgccagtccccaacgaaatctt

SEQ ID NO: 23 - DNA, 25 bp, synthetic construct
  source 1..25: mol_type = other DNA
  misc_feature 12: note = LNA
  misc_feature 14: note = LNA
  misc_feature 25: note = LNA
gttcaaggacttggtccaggttgta

SEQ ID NO: 24 - DNA, 25 bp, synthetic construct
  source 1..25: mol_type = other DNA
  misc_feature 1: note = LNA
  misc_feature 12: note = LNA
  misc_feature 14: note = LNA
  misc_feature 25: note = LNA
gttcaaggacttggtccaggttgta

SEQ ID NO: 25 - DNA, 25 bp, synthetic construct
  source 1..25: mol_type = other DNA
  misc_feature 1..2: note = LNA
  misc_feature 12: note = LNA
  misc_feature 14: note = LNA
gttcaaggacttggtccaggttgta

SEQ ID NO: 26 - DNA, 25 bp, synthetic construct
  source 1..25: mol_type = other DNA
  misc_feature 1..3: note = LNA
  misc_feature 12: note = LNA
  misc_feature 14: note = LNA
gttcaaggacttggtccaggttgta

SEQ ID NO: 27 - DNA, 25 bp, synthetic construct
  source 1..25: mol_type = other DNA
  misc_feature 1..2: note = LNA
  misc_feature 12: note = LNA
  misc_feature 14: note = LNA
  misc_feature 25: note = LNA
gttcaaggacttggtccaggttgta

SEQ ID NO: 28 - DNA, 25 bp, synthetic construct
  source 1..25: mol_type = other DNA
  misc_feature 1: note = LNA
  misc_feature 12: note = LNA
  misc_feature 14: note = LNA
  misc_feature 24..25: note = LNA
gttcaaggacttggtccaggttgta

SEQ ID NO: 29 - DNA, 25 bp, synthetic construct
  source 1..25: mol_type = other DNA
  misc_feature 1: note = LNA
  misc_feature 12: note = LNA
  misc_feature 14: note = LNA
  misc_feature 23..25: note = LNA
gttcaaggacttggtccaggttgta

SEQ ID NO: 30 - DNA, 25 bp, synthetic construct
  source 1..25: mol_type = other DNA
  misc_feature 1: note = LNA
  misc_feature 12: note = LNA
  misc_feature 14: note = LNA
  misc_feature 1..2: note = Phosphorothioate linkage
gttcaaggacttggtccaggttgta

SEQ ID NO: 31 - DNA, 25 bp, synthetic construct
  source 1..25: mol_type = other DNA
  misc_feature 1: note = LNA
  misc_feature 12: note = LNA
  misc_feature 14: note = LNA
  misc_feature 1..3: note = Phosphorothioate linkage
gttcaaggacttggtccaggttgta

SEQ ID NO: 32 - DNA, 25 bp, synthetic construct
  source 1..25: mol_type = other DNA
  misc_feature 1: note = LNA
  misc_feature 12: note = LNA
  misc_feature 14: note = LNA
  misc_feature 1..4: note = Phosphorothioate linkage
gttcaaggacttggtccaggttgta

SEQ ID NO: 33 - DNA, 25 bp, synthetic construct
  source 1..25: mol_type = other DNA
  misc_feature 1: note = LNA
  misc_feature 12: note = LNA
  misc_feature 14: note = LNA
  misc_feature 1..5: note = Phosphorothioate linkage
gttcaaggacttggtccaggttgta

SEQ ID NO: 34 - DNA, 25 bp, synthetic construct
  source 1..25: mol_type = other DNA
  misc_feature 1: note = LNA
  misc_feature 12: note = LNA
  misc_feature 14: note = LNA
  misc_feature 1..6: note = Phosphorothioate linkage
gttcaaggacttggtccaggttgta

SEQ ID NO: 35 - DNA, 25 bp, synthetic construct
  source 1..25: mol_type = other DNA
  misc_feature 1: note = LNA
  misc_feature 12: note = LNA
  misc_feature 14: note = LNA
  misc_feature 24..25: note = Phosphorothioate linkage
gttcaaggacttggtccaggttgta

SEQ ID NO: 36 - DNA, 25 bp, synthetic construct
  source 1..25: mol_type = other DNA
  misc_feature 1: note = LNA
  misc_feature 12: note = LNA
  misc_feature 14: note = LNA
  misc_feature 23..25: note = Phosphorothioate linkage
gttcaaggacttggtccaggttgta

SEQ ID NO: 37 - DNA, 25 bp, synthetic construct
  source 1..25: mol_type = other DNA
  misc_feature 1: note = LNA
  misc_feature 12: note = LNA
  misc_feature 14: note = LNA
  misc_feature 22..25: note = Phosphorothioate linkage
gttcaaggacttggtccaggttgta

SEQ ID NO: 38 - DNA, 25 bp, synthetic construct
  source 1..25: mol_type = other DNA
  misc_feature 1: note = LNA
  misc_feature 12: note = LNA
  misc_feature 14: note = LNA
  misc_feature 21..25: note = Phosphorothioate linkage
gttcaaggacttggtccaggttgta

SEQ ID NO: 39 - DNA, 25 bp, synthetic construct
  source 1..25: mol_type = other DNA
  misc_feature 1: note = LNA
  misc_feature 12: note = LNA
  misc_feature 14: note = LNA
  misc_feature 20..25: note = Phosphorothioate linkage
gttcaaggacttggtccaggttgta

SEQ ID NO: 40 - DNA, 25 bp, synthetic construct
  source 1..25: mol_type = other DNA
  misc_feature 1: note = LNA
  misc_feature 12: note = LNA
  misc_feature 14: note = LNA
  misc_feature 19..25: note = Phosphorothioate linkage
gttcaaggacttggtccaggttgta

SEQ ID NO: 41 - DNA, 25 bp, synthetic construct
  source 1..25: mol_type = other DNA
  misc_feature 1: note = LNA
  misc_feature 12: note = LNA
  misc_feature 14: note = LNA
  misc_feature 18..25: note = Phosphorothioate linkage
gttcaaggacttggtccaggttgta

SEQ ID NO: 42 - DNA, 25 bp, synthetic construct
  source 1..25: mol_type = other DNA
  misc_feature 1: note = LNA
  misc_feature 12: note = LNA
  misc_feature 14: note = LNA
  misc_feature 1..5: note = Phosphorothioate linkage
  misc_feature 21..25: note = Phosphorothioate linkage
gttcaaggacttggtccaggttgta

SEQ ID NO: 43 - DNA, 25 bp, synthetic construct
  source 1..25: mol_type = other DNA
  misc_feature 1: note = LNA
  misc_feature 12: note = LNA
  misc_feature 14: note = LNA
  misc_feature 10..12: note = Phosphorothioate linkage
gttcaaggacttggtccaggttgta

SEQ ID NO: 44 - DNA, 25 bp, synthetic construct
  source 1..25: mol_type = other DNA
  misc_feature 1: note = LNA
  misc_feature 12: note = LNA
  misc_feature 14: note = LNA
  misc_feature 8..12: note = Phosphorothioate linkage
gttcaaggacttggtccaggttgta

SEQ ID NO: 45 - DNA, 25 bp, synthetic construct
  source 1..25: mol_type = other DNA
  misc_feature 1: note = LNA
  misc_feature 12: note = LNA
  misc_feature 14: note = LNA
  misc_feature 15..17: note = Phosphorothioate linkage
gttcaaggacttggtccaggttgta

SEQ ID NO: 46 - DNA, 25 bp, synthetic construct
  source 1..25: mol_type = other DNA
  misc_feature 1: note = LNA
  misc_feature 12: note = LNA
  misc_feature 14: note = LNA
  misc_feature 15..19: note = Phosphorothioate linkage
gttcaaggacttggtccaggttgta

SEQ ID NO: 47 - DNA, 25 bp, synthetic construct
  source 1..25: mol_type = other DNA
  misc_feature 1: note = LNA
  misc_feature 12: note = LNA
  misc_feature 14: note = LNA
  misc_feature 25: note = LNA
  misc_feature 24..25: note = Phosphorothioate linkage
gttcaaggacttggtccaggttgta

SEQ ID NO: 48 - DNA, 25 bp, synthetic construct
  source 1..25: mol_type = other DNA
  misc_feature 1: note = LNA
  misc_feature 12: note = LNA
  misc_feature 14: note = LNA
  misc_feature 25: note = LNA
  misc_feature 23..25: note = Phosphorothioate linkage
gttcaaggacttggtccaggttgta

SEQ ID NO: 49 - DNA, 25 bp, synthetic construct
  source 1..25: mol_type = other DNA
  misc_feature 1: note = LNA
  misc_feature 12: note = LNA
  misc_feature 14: note = LNA
  misc_feature 25: note = LNA
  misc_feature 22..25: note = Phosphorothioate linkage
gttcaaggacttggtccaggttgta

SEQ ID NO: 50 - DNA, 25 bp, synthetic construct
  source 1..25: mol_type = other DNA
  misc_feature 1: note = LNA
  misc_feature 12: note = LNA
  misc_feature 14: note = LNA
  misc_feature 25: note = LNA
  misc_feature 21..25: note = Phosphorothioate linkage
gttcaaggacttggtccaggttgta

SEQ ID NO: 51 - DNA, 38 bp, synthetic construct
  source 1..38: mol_type = other DNA
  misc_feature 1: note = LNA
  misc_feature 25: note = LNA
  misc_feature 27: note = LNA
gacacacctccctgttcaaggacttggtccaggttgta

SEQ ID NO: 52 - DNA, 38 bp, synthetic construct; identical to SEQ ID NO: 51
  source 1..38: mol_type = other DNA
  misc_feature 1: note = LNA
  misc_feature 14: note = LNA
  misc_feature 25: note = LNA
  misc_feature 27: note = LNA

SEQ ID NO: 53 - DNA, 38 bp, synthetic construct; identical to SEQ ID NO: 51
  source 1..38: mol_type = other DNA
  misc_feature 1..2: note = LNA
  misc_feature 25: note = LNA
  misc_feature 27: note = LNA

SEQ ID NO: 54 - DNA, 38 bp, synthetic construct; identical to SEQ ID NO: 51
  source 1..38: mol_type = other DNA
  misc_feature 1..2: note = LNA
  misc_feature 14: note = LNA
  misc_feature 25: note = LNA
  misc_feature 27: note = LNA

SEQ ID NO: 55 - DNA, 38 bp, synthetic construct; identical to SEQ ID NO: 51
  source 1..38: mol_type = other DNA
  misc_feature 1..3: note = LNA
  misc_feature 25: note = LNA
  misc_feature 27: note = LNA

SEQ ID NO: 56 - DNA, 38 bp, synthetic construct; identical to SEQ ID NO: 51
  source 1..38: mol_type = other DNA
  misc_feature 1..3: note = LNA
  misc_feature 14: note = LNA
  misc_feature 25: note = LNA
  misc_feature 27: note = LNA

SEQ ID NO: 57 - DNA, 40 bp, synthetic construct
  source 1..40: mol_type = other DNA
  misc_feature 1: note = LNA
  misc_feature 12: note = LNA
  misc_feature 14: note = LNA
  misc_feature 40: note = LNA
gttcaaggacttggtccaggttgtagccggctgtctgtcg

SEQ ID NO: 58 - DNA, 40 bp, synthetic construct; identical to SEQ ID NO: 57
  source 1..40: mol_type = other DNA
  misc_feature 1: note = LNA
  misc_feature 12: note = LNA
  misc_feature 14: note = LNA
  misc_feature 25: note = LNA
  misc_feature 40: note = LNA

SEQ ID NO: 59 - DNA, 40 bp, synthetic construct; identical to SEQ ID NO: 57
  source 1..40: mol_type = other DNA
  misc_feature 1: note = LNA
  misc_feature 12: note = LNA
  misc_feature 14: note = LNA
  misc_feature 39..40: note = LNA

SEQ ID NO: 60 - DNA, 40 bp, synthetic construct; identical to SEQ ID NO: 57
  source 1..40: mol_type = other DNA
  misc_feature 1: note = LNA
  misc_feature 12: note = LNA
  misc_feature 14: note = LNA
  misc_feature 25: note = LNA
  misc_feature 39..40: note = LNA

SEQ ID NO: 61 - DNA, 40 bp, synthetic construct; identical to SEQ ID NO: 57
  source 1..40: mol_type = other DNA
  misc_feature 1: note = LNA
  misc_feature 12: note = LNA
  misc_feature 14: note = LNA
  misc_feature 38..40: note = LNA

SEQ ID NO: 62 - DNA, 40 bp, synthetic construct; identical to SEQ ID NO: 57
  source 1..40: mol_type = other DNA
  misc_feature 1: note = LNA
  misc_feature 12: note = LNA
  misc_feature 14: note = LNA
  misc_feature 25: note = LNA
  misc_feature 38..40: note = LNA

SEQ ID NO: 63 - DNA, 25 bp, synthetic construct
  source 1..25: mol_type = other DNA
  misc_feature 1: note = LNA
  misc_feature 12: note = LNA
  misc_feature 14: note = LNA
  misc_feature 25: note = LNA
  misc_feature 24: note = Ribonucleotide
gttcaaggacttggtccaggttgta

SEQ ID NO: 64 - DNA, 25 bp, synthetic construct
  source 1..25: mol_type = other DNA
  misc_feature 1: note = LNA
  misc_feature 12: note = LNA
  misc_feature 14: note = LNA
  misc_feature 25: note = LNA
  misc_feature 23..24: note = Ribonucleotide
gttcaaggacttggtccaggttgta

SEQ ID NO: 65 - DNA, 25 bp, synthetic construct
  source 1..25: mol_type = other DNA
  misc_feature 1: note = LNA
  misc_feature 12: note = LNA
  misc_feature 14: note = LNA
  misc_feature 25: note = LNA
  misc_feature 22..24: note = Ribonucleotide
gttcaaggacttggtccaggttgta

SEQ ID NO: 66 - DNA, 25 bp, synthetic construct
  source 1..25: mol_type = other DNA
  misc_feature 1: note = LNA
  misc_feature 12: note = LNA
  misc_feature 14: note = LNA
  misc_feature 25: note = LNA
  misc_feature 21..24: note = Ribonucleotide
gttcaaggacttggtccaggttgta

SEQ ID NO: 67 - DNA, 25 bp, synthetic construct
  source 1..25: mol_type = other DNA
  misc_feature 1: note = LNA
  misc_feature 12: note = LNA
  misc_feature 14: note = LNA
  misc_feature 1: note = 5' phosphate
gttcaaggacttggtccaggttgta

SEQ ID NO: 68 - DNA, 25 bp, synthetic construct
  source 1..25: mol_type = other DNA
  misc_feature 1: note = LNA
  misc_feature 12: note = LNA
  misc_feature 14: note = LNA
  misc_feature 25: note = 3' phosphate
gttcaaggacttggtccaggttgta

SEQ ID NO: 69 - DNA, 25 bp, synthetic construct
  source 1..25: mol_type = other DNA
  misc_feature 1: note = LNA
  misc_feature 12: note = LNA
  misc_feature 14: note = LNA
  misc_feature 1: note = 5' phosphate
  misc_feature 25: note = 3' phosphate
gttcaaggacttggtccaggttgta

SEQ ID NO: 70 - DNA, 25 bp, synthetic construct
  source 1..25: mol_type = other DNA
  misc_feature 1: note = LNA
  misc_feature 12: note = LNA
  misc_feature 14: note = LNA
  misc_feature 25: note = LNA
  misc_feature 25: note = 3' phosphate
gttcaaggacttggtccaggttgta

SEQ ID NO: 71 - DNA, 25 bp, synthetic construct
  source 1..25: mol_type = other DNA
  misc_feature 1: note = LNA
  misc_feature 12: note = LNA
  misc_feature 14: note = LNA
  misc_feature 25: note = LNA
  misc_feature 24..25: note = Phosphorothioate linkage
  misc_feature 25: note = 3' phosphate
gttcaaggacttggtccaggttgta

SEQ ID NO: 72 - DNA, 25 bp, synthetic construct
  source 1..25: mol_type = other DNA
  misc_feature 1: note = BNA-N-H
  misc_feature 12: note = LNA
  misc_feature 14: note = LNA
gttcaaggacttggtccaggttgta

SEQ ID NO: 73 - DNA, 25 bp, synthetic construct
  source 1..25: mol_type = other DNA
  misc_feature 1: note = BNA-N-Me
  misc_feature 12: note = LNA
  misc_feature 14: note = LNA
gttcaaggacttggtccaggttgta

SEQ ID NO: 74 - DNA, 25 bp, synthetic construct
  source 1..25: mol_type = other DNA
  misc_feature 1: note = ENA
  misc_feature 12: note = LNA
  misc_feature 14: note = LNA
gttcaaggacttggtccaggttgta

SEQ ID NO: 75 - DNA, 25 bp, synthetic construct
  source 1..25: mol_type = other DNA
  misc_feature 1: note = LNA
  misc_feature 12: note = LNA
  misc_feature 14: note = LNA
  misc_feature 20..25: note = Phosphorothioate linkage
  misc_feature 25: note = 3' phosphate
gttcaaggacttggtccaggttgta

SEQ ID NO: 76 - DNA, 29 bp, synthetic construct
  source 1..29: mol_type = other DNA
  misc_feature 1: note = LNA
  misc_feature 14: note = LNA
  misc_feature 16: note = LNA
  misc_feature 29: note = LNA
  misc_feature 1..5: note = Phosphorothioate linkage
  misc_feature 27..28: note = Ribonucleotide
  misc_feature 29: note = 3' phosphate
ctgttcaaggacttggtccaggttgtagc

SEQ ID NO: 77 - DNA, 35 bp, synthetic construct
  source 1..35: mol_type = other DNA
tagccggctgtctgtcgccagtccccaacgaaatc

SEQ ID NO: 78 - DNA, 35 bp, synthetic construct; identical to SEQ ID NO: 77
  source 1..35: mol_type = other DNA
  misc_feature 16..19: note = LNA

SEQ ID NO: 79 - DNA, 35 bp, synthetic construct; identical to SEQ ID NO: 77
  source 1..35: mol_type = other DNA
  misc_feature 1: note = LNA
  misc_feature 16..19: note = LNA

SEQ ID NO: 80 - DNA, 39 bp, synthetic construct
  source 1..39: mol_type = other DNA
  misc_feature 1: note = LNA
  misc_feature 25..28: note = LNA
tccaggttgtagccggctgtctgtcgccagtccccaacg

SEQ ID NO: 81 - DNA, 39 bp, synthetic construct; identical to SEQ ID NO: 80
  source 1..39: mol_type = other DNA
  misc_feature 34..39: note = Phosphorothioate linkage
  misc_feature 1..3: note = LNA
  misc_feature 25..27: note = LNA

SEQ ID NO: 82 - DNA, 39 bp, synthetic construct; identical to SEQ ID NO: 80
  source 1..39: mol_type = other DNA
  misc_feature 34..39: note = Phosphorothioate linkage
  misc_feature 1..3: note = LNA
  misc_feature 26..27: note = LNA

SEQ ID NO: 83 - DNA, 36 bp, synthetic construct
  source 1..36: mol_type = other DNA
gacaccccgagattctgaaacaaactggacacacct

SEQ ID NO: 84 - DNA, 36 bp, synthetic construct; identical to SEQ ID NO: 83
  source 1..36: mol_type = other DNA
  misc_feature 16..20: note = LNA

SEQ ID NO: 85 - DNA, 36 bp, synthetic construct; identical to SEQ ID NO: 83
  source 1..36: mol_type = other DNA
  misc_feature 1: note = LNA
  misc_feature 16..20: note = LNA

SEQ ID NO: 86 - DNA, 40 bp, synthetic construct
  source 1..40: mol_type = other DNA
  misc_feature 1: note = LNA
  misc_feature 25..29: note = LNA
ggagttacggacaccccgagattctgaaacaaactggaca

SEQ ID NO: 87 - DNA, 40 bp, synthetic construct; identical to SEQ ID NO: 86
  source 1..40: mol_type = other DNA
  misc_feature 35..40: note = Phosphorothioate linkage
  misc_feature 1..3: note = LNA
  misc_feature 25..29: note = LNA

SEQ ID NO: 88 - DNA, 47 bp, synthetic construct
  source 1..47: mol_type = other DNA
aacaaactggacacacctcactgttcaaggacttggtccaggttgta

SEQ ID NO: 89 - DNA, 47 bp, synthetic construct; identical to SEQ ID NO: 88
  source 1..47: mol_type = other DNA
  misc_feature 25: note = LNA
  misc_feature 27: note = LNA
  misc_feature 34: note = LNA
  misc_feature 36: note = LNA

SEQ ID NO: 90 - DNA, 47 bp, synthetic construct; identical to SEQ ID NO: 88
  source 1..47: mol_type = other DNA
  misc_feature 1: note = LNA
  misc_feature 25: note = LNA
  misc_feature 27: note = LNA
  misc_feature 34: note = LNA
  misc_feature 36: note = LNA

SEQ ID NO: 91 - DNA, 47 bp, synthetic construct; identical to SEQ ID NO: 88
  source 1..47: mol_type = other DNA
  misc_feature 42..47: note = Phosphorothioate linkage
  misc_feature 1..3: note = LNA
  misc_feature 25: note = LNA
  misc_feature 27: note = LNA
  misc_feature 34: note = LNA
  misc_feature 36: note = LNA

SEQ ID NO: 92 - DNA, 53 bp, synthetic construct
  source 1..53: mol_type = other DNA
ttctaaaacaaactggacacacctccctgttaaaggacttggtccaggttgta

SEQ ID NO: 93 - DNA, 53 bp, synthetic construct; identical to SEQ ID NO: 92
  source 1..53: mol_type = other DNA
  misc_feature 25: note = LNA
  misc_feature 27: note = LNA
  misc_feature 40: note = LNA
  misc_feature 42: note = LNA

SEQ ID NO: 94 - DNA, 53 bp, synthetic construct; identical to SEQ ID NO: 92
  source 1..53: mol_type = other DNA
  misc_feature 1: note = LNA
  misc_feature 25: note = LNA
  misc_feature 27: note = LNA
  misc_feature 40: note = LNA
  misc_feature 42: note = LNA

SEQ ID NO: 95 - DNA, 53 bp, synthetic construct; identical to SEQ ID NO: 92
  source 1..53: mol_type = other DNA
  misc_feature 48..53: note = Phosphorothioate linkage
  misc_feature 1..3: note = LNA
  misc_feature 25: note = LNA
  misc_feature 27: note = LNA
  misc_feature 40: note = LNA
  misc_feature 42: note = LNA

SEQ ID NO: 96 - DNA, 59 bp, synthetic construct
  source 1..59: mol_type = other DNA
ggagttacggacaccccgagattctgaaacaaactggacacacctccctgttaaaggac

SEQ ID NO: 97 - DNA, 59 bp, synthetic construct; identical to SEQ ID NO: 96
  source 1..59: mol_type = other DNA
  misc_feature 25: note = LNA
  misc_feature 27: note = LNA
  misc_feature 46: note = LNA
  misc_feature 48: note = LNA

SEQ ID NO: 98 - DNA, 59 bp, synthetic construct; identical to SEQ ID NO: 96
  source 1..59: mol_type = other DNA
  misc_feature 1: note = LNA
  misc_feature 25: note = LNA
  misc_feature 27: note = LNA
  misc_feature 46: note = LNA
  misc_feature 48: note = LNA

SEQ ID NO: 99 - DNA, 59 bp, synthetic construct; identical to SEQ ID NO: 96
  source 1..59: mol_type = other DNA
  misc_feature 54..59: note = Phosphorothioate linkage
  misc_feature 1..3: note = LNA
  misc_feature 25: note = LNA
  misc_feature 27: note = LNA
  misc_feature 46: note = LNA
  misc_feature 48: note = LNA

SEQ ID NO: 100 - DNA, 35 bp, synthetic construct
  source 1..35: mol_type = other DNA
tcctttggatcggagttacggacaccccgagattc

SEQ ID NO: 101 - DNA, 35 bp, synthetic construct; identical to SEQ ID NO: 100
  source 1..35: mol_type = other DNA
  misc_feature 18: note = LNA
  misc_feature 20: note = LNA

SEQ ID NO: 102 - DNA, 38 bp, synthetic construct
  source 1..38: mol_type = other DNA
  misc_feature 1: note = LNA
  misc_feature 25: note = LNA
  misc_feature 27: note = LNA
aggacaatcctttggatcggagttacggacaccccgag

SEQ ID NO: 103 - DNA, 38 bp, synthetic construct; identical to SEQ ID NO: 102
  source 1..38: mol_type = other DNA
  misc_feature 33..38: note = Phosphorothioate linkage
  misc_feature 1..3: note = LNA
  misc_feature 25: note = LNA
  misc_feature 27: note = LNA

SEQ ID NO: 104 - DNA, 38 bp, synthetic construct; identical to SEQ ID NO: 102
  source 1..38: mol_type = other DNA
  misc_feature 33..38: note = Phosphorothioate linkage
  misc_feature 1..3: note = LNA
  misc_feature 25..27: note = LNA

SEQ ID NO: 105 - DNA, 39 bp, synthetic construct
  source 1..39: mol_type = other DNA
cctgttcaaggacttggtccaggttgtagccggctgtct

SEQ ID NO: 106 - DNA, 39 bp, synthetic construct; identical to SEQ ID NO: 105
  source 1..39: mol_type = other DNA
  misc_feature 25: note = LNA
  misc_feature 28: note = LNA

SEQ ID NO: 107 - DNA, 39 bp, synthetic construct; identical to SEQ ID NO: 105
  source 1..39: mol_type = other DNA
  misc_feature 1: note = LNA
  misc_feature 25: note = LNA
  misc_feature 28: note = LNA

SEQ ID NO: 108 - DNA, 39 bp, synthetic construct; identical to SEQ ID NO: 105
  source 1..39: mol_type = other DNA
  misc_feature 34..39: note = Phosphorothioate linkage
  misc_feature 1..3: note = LNA
  misc_feature 25: note = LNA
  misc_feature 28: note = LNA

SEQ ID NO: 109 - DNA, 39 bp, synthetic construct; identical to SEQ ID NO: 105
  source 1..39: mol_type = other DNA
  misc_feature 34..39: note = Phosphorothioate linkage
  misc_feature 1..3: note = LNA
  misc_feature 25..28: note = LNA

SEQ ID NO: 110 - DNA, 39 bp, synthetic construct; identical to SEQ ID NO: 105
  source 1..39: mol_type = other DNA
  misc_feature 34..39: note = Phosphorothioate linkage
  misc_feature 1..3: note = LNA
  misc_feature 25..27: note = LNA

SEQ ID NO: 111 - DNA, 39 bp, synthetic construct; identical to SEQ ID NO: 105
  source 1..39: mol_type = other DNA
  misc_feature 34..39: note = Phosphorothioate linkage
  misc_feature 1..3: note = LNA
  misc_feature 25..26: note = LNA
  misc_feature 28: note = LNA

SEQ ID NO: 112 - DNA, 39 bp, synthetic construct; identical to SEQ ID NO: 105
  source 1..39: mol_type = other DNA
  misc_feature 34..39: note = Phosphorothioate linkage
  misc_feature 1..3: note = LNA
  misc_feature 25: note = LNA
  misc_feature 27..28: note = LNA

SEQ ID NO: 113 - DNA, 39 bp, synthetic construct; identical to SEQ ID NO: 105
  source 1..39: mol_type = other DNA
  misc_feature 34..39: note = Phosphorothioate linkage
  misc_feature 1..3: note = LNA
  misc_feature 26..28: note = LNA

SEQ ID NO: 114 - DNA, 39 bp, synthetic construct; identical to SEQ ID NO: 105
  source 1..39: mol_type = other DNA
  misc_feature 34..39: note = Phosphorothioate linkage
  misc_feature 1..3: note = LNA
  misc_feature 26..27: note = LNA

SEQ ID NO: 115 - DNA, 37 bp, synthetic construct
  source 1..37: mol_type = other DNA
acaaactggacacacctccctgttcaaggacttggtc

SEQ ID NO: 116 - DNA, 37 bp, synthetic construct; identical to SEQ ID NO: 115
  source 1..37: mol_type = other DNA
  misc_feature 25..26: note = LNA

SEQ ID NO: 117 - DNA, 37 bp, synthetic construct; identical to SEQ ID NO: 115
  source 1..37: mol_type = other DNA
  misc_feature 1: note = LNA
  misc_feature 25..26: note = LNA

SEQ ID NO: 118 - DNA, 37 bp, synthetic construct; identical to SEQ ID NO: 115
  source 1..37: mol_type = other DNA
  misc_feature 32..37: note = Phosphorothioate linkage
  misc_feature 1..3: note = LNA
  misc_feature 25..26: note = LNA

SEQ ID NO: 119 - DNA, 37 bp, synthetic construct
  source 1..37: mol_type = other DNA
tcaggacaatcctttggatcggagttacggacacccc

SEQ ID NO: 120 - DNA, 37 bp, synthetic construct; identical to SEQ ID NO: 119
  source 1..37: mol_type = other DNA
  misc_feature 25..26: note = LNA

SEQ ID NO: 121 - DNA, 37 bp, synthetic construct; identical to SEQ ID NO: 119
  source 1..37: mol_type = other DNA
  misc_feature 1: note = LNA
  misc_feature 25..26: note = LNA

SEQ ID NO: 122 - DNA, 37 bp, synthetic construct; identical to SEQ ID NO: 119
  source 1..37: mol_type = other DNA
  misc_feature 32..37: note = Phosphorothioate linkage
  misc_feature 1..3: note = LNA
  misc_feature 25..26: note = LNA

SEQ ID NO: 123 - DNA, 39 bp, synthetic construct
  source 1..39: mol_type = other DNA
tcctttggatcggagttacggacaccccgagattctgaa

SEQ ID NO: 124 - DNA, 39 bp, synthetic construct; identical to SEQ ID NO: 123
  source 1..39: mol_type = other DNA
  misc_feature 18: note = LNA
  misc_feature 23: note = LNA

SEQ ID NO: 125 - DNA, 39 bp, synthetic construct; identical to SEQ ID NO: 123
  source 1..39: mol_type = other DNA
  misc_feature 1: note = LNA
  misc_feature 18: note = LNA
  misc_feature 23: note = LNA

SEQ ID NO: 126 - DNA, 41 bp, synthetic construct
  source 1..41: mol_type = other DNA
  misc_feature 1: note = LNA
  misc_feature 25: note = LNA
  misc_feature 30: note = LNA
aggacaatcctttggatcggagttacggacaccccgagatt

SEQ ID NO: 127 - DNA, 41 bp, synthetic construct; identical to SEQ ID NO: 126
  source 1..41: mol_type = other DNA
  misc_feature 36..41: note = Phosphorothioate linkage
  misc_feature 1..3: note = LNA
  misc_feature 25: note = LNA
  misc_feature 30: note = LNA

SEQ ID NO: 128 - DNA, 25 bp, synthetic construct
  source 1..25: mol_type = other DNA
  misc_feature 20..25: note = Phosphorothioate linkage
  misc_feature 25: note = 3' phosphate
  misc_feature 1: note = LNA
  misc_feature 12: note = LNA
  misc_feature 14: note = LNA
gttcaaggacttggtccaggttgta

SEQ ID NO: 129 - DNA, 25 bp, synthetic construct
  source 1..25: mol_type = other DNA
  misc_feature 14..25: note = Phosphorothioate linkage
  misc_feature 1: note = LNA
  misc_feature 12: note = LNA
  misc_feature 14: note = LNA
gttcaaggacttggtccaggttgta

SEQ ID NO: 130 - DNA, 25 bp, synthetic construct
  misc_feature 24: note = Ribonucleotide
  source 1..25: mol_type = other DNA
  misc_feature 24..25: note = Phosphorothioate linkage
  misc_feature 1: note = LNA
  misc_feature 12: note = LNA
  misc_feature 14: note = LNA
  misc_feature 25: note = LNA
gttcaaggacttggtccaggttgta

SEQ ID NO: 131 - DNA, 25 bp, synthetic construct
  source 1..25: mol_type = other DNA
  misc_feature 22..25: note = Phosphorothioate linkage
  misc_feature 23: note = 2'-Fluoro-modified
  misc_feature 24: note = 2'-Fluoro-modified
  misc_feature 1: note = LNA
  misc_feature 12: note = LNA
  misc_feature 14: note = LNA
  misc_feature 23..25: note = LNA
gttcaaggacttggtccaggttgta

SEQ ID NO: 132 - DNA, 25 bp, synthetic construct
  source 1..25: mol_type = other DNA
  misc_feature 23..25: note = Phosphorothioate linkage
  misc_feature 25: note = 2'-O-Methyl-modified
  misc_feature 1: note = LNA
  misc_feature 12: note = LNA
  misc_feature 14: note = LNA
  misc_feature 25: note = LNA
gttcaaggacttggtccaggttgta

SEQ ID NO: 133 - DNA, 25 bp, synthetic construct
  source 1..25: mol_type = other DNA
  misc_feature 1..3: note = Phosphorothioate linkage
  misc_feature 24..25: note = Phosphorothioate linkage
  misc_feature 1: note = LNA
  misc_feature 12: note = LNA
  misc_feature 14: note = LNA
  misc_feature 25: note = LNA
gttcaaggacttggtccaggttgta

SEQ ID NO: 134 - DNA, 25 bp, synthetic construct
  source 1..25: mol_type = other DNA
  misc_feature 1..3: note = Phosphorothioate linkage
  misc_feature 22..25: note = Phosphorothioate linkage
  misc_feature 1: note = LNA
  misc_feature 12: note = LNA
  misc_feature 14: note = LNA
  misc_feature 25: note = LNA
gttcaaggacttggtccaggttgta

SEQ ID NO: 135 - DNA, 25 bp, synthetic construct
  source 1..25: mol_type = other DNA
  misc_feature 1..3: note = Phosphorothioate linkage
  misc_feature 24..25: note = Phosphorothioate linkage
  misc_feature 1: note = LNA
  misc_feature 12: note = LNA
  misc_feature 14: note = LNA
gttcaaggacttggtccaggttgta

SEQ ID NO: 136 - DNA, 25 bp, synthetic construct
  source 1..25: mol_type = other DNA
  misc_feature 1..3: note = Phosphorothioate linkage
  misc_feature 23..25: note = Phosphorothioate linkage
  misc_feature 1: note = LNA
  misc_feature 12: note = LNA
  misc_feature 14: note = LNA
  misc_feature 25: note = LNA
gttcaaggacttggtccaggttgta

SEQ ID NO: 137 - DNA, 25 bp, synthetic construct
  source 1..25: mol_type = other DNA
  misc_feature 1..3: note = Phosphorothioate linkage
  misc_feature 20..25: note = Phosphorothioate linkage
  misc_feature 1: note = LNA
  misc_feature 12: note = LNA
  misc_feature 14: note = LNA
gttcaaggacttggtccaggttgta

SEQ ID NO: 138 - DNA, 25 bp, synthetic construct
  misc_feature 2..3: note = Ribonucleotide
  source 1..25: mol_type = other DNA
  misc_feature 1..5: note = Phosphorothioate linkage
  misc_feature 22..25: note = Phosphorothioate linkage
  misc_feature 1: note = LNA
  misc_feature 12: note = LNA
  misc_feature 14: note = LNA
  misc_feature 25: note = LNA
gttcaaggacttggtccaggttgta

SEQ ID NO: 139 - DNA, 25 bp, synthetic construct
  misc_feature 2..3: note = Ribonucleotide
  source 1..25: mol_type = other DNA
  misc_feature 1..5: note = Phosphorothioate linkage
  misc_feature 24..25: note = Phosphorothioate linkage
  misc_feature 1: note = LNA
  misc_feature 12: note = LNA
  misc_feature 14: note = LNA
gttcaaggacttggtccaggttgta

SEQ ID NO: 140 - DNA, 25 bp, synthetic construct
  misc_feature 2..3: note = Ribonucleotide
  source 1..25: mol_type = other DNA
  misc_feature 1..5: note = Phosphorothioate linkage
  misc_feature 23..25: note = Phosphorothioate linkage
  misc_feature 1: note = LNA
  misc_feature 12: note = LNA
  misc_feature 14: note = LNA
  misc_feature 25: note = LNA
gttcaaggacttggtccaggttgta

SEQ ID NO: 141 - DNA, 25 bp, synthetic construct
  source 1..25: mol_type = other DNA
  misc_feature 1..3: note = Phosphorothioate linkage
  misc_feature 24..25: note = Phosphorothioate linkage
  misc_feature 25: note = 3' phosphate
  misc_feature 1: note = LNA
  misc_feature 12: note = LNA
  misc_feature 14: note = LNA
gttcaaggacttggtccaggttgta

SEQ ID NO: 142 - DNA, 38 bp, synthetic construct; identical to SEQ ID NO: 51
  source 1..38: mol_type = other DNA
  misc_feature 33..38: note = Phosphorothioate linkage
  misc_feature 1..3: note = LNA
  misc_feature 25: note = LNA
  misc_feature 27: note = LNA

SEQ ID NO: 143 - DNA, 38 bp, synthetic construct; identical to SEQ ID NO: 51
  source 1..38: mol_type = other DNA
  misc_feature 33..38: note = Phosphorothioate linkage
  misc_feature 38: note = 3' phosphate
  misc_feature 1..3: note = LNA
  misc_feature 25: note = LNA
  misc_feature 27: note = LNA

SEQ ID NO: 144 - DNA, 25 bp, synthetic construct
  source 1..25: mol_type = other DNA
  misc_feature 24..25: note = Methylphosphate linkage
  misc_feature 1: note = LNA
  misc_feature 12: note = LNA
  misc_feature 14: note = LNA
gttcaaggacttggtccaggttgta

SEQ ID NO: 145 - DNA, 28 bp, synthetic construct
  source 1..28: mol_type = other DNA
  misc_feature 1: note = LNA
  misc_feature 12: note = LNA
  misc_feature 14: note = LNA
gttcaaggacttggtccaggttgtatat

SEQ ID NO: 146 - DNA, 28 bp, synthetic construct
  source 1..28: mol_type = other DNA
  misc_feature 1: note = LNA
  misc_feature 12: note = LNA
  misc_feature 14: note = LNA
  misc_feature 28: note = LNA
gttcaaggacttggtccaggttgtatat

SEQ ID NO: 147 - DNA, 28 bp, synthetic construct
  source 1..28: mol_type = other DNA
  misc_feature 23..28: note = Phosphorothioate linkage
  misc_feature 1: note = LNA
  misc_feature 12: note = LNA
  misc_feature 14: note = LNA
gttcaaggacttggtccaggttgtatat

SEQ ID NO: 148 - DNA, 28 bp, synthetic construct
  misc_feature 26..28: note = Ribonucleotide
  source 1..28: mol_type = other DNA
  misc_feature 23..28: note = Phosphorothioate linkage
  misc_feature 1: note = LNA
  misc_feature 12: note = LNA
  misc_feature 14: note = LNA
gttcaaggacttggtccaggttgtatat

SEQ ID NO: 149 - DNA, 28 bp, synthetic construct
  source 1..28: mol_type = other DNA
  misc_feature 23..28: note = Phosphorothioate linkage
  misc_feature 1: note = LNA
  misc_feature 12: note = LNA
  misc_feature 14: note = LNA
  misc_feature 28: note = LNA
gttcaaggacttggtccaggttgtatat

SEQ ID NO: 150 - DNA, 31 bp, synthetic construct
  source 1..31: mol_type = other DNA
  misc_feature 1: note = LNA
  misc_feature 12: note = LNA
  misc_feature 14: note = LNA
gttcaaggacttggtccaggttgtatatata

SEQ ID NO: 151 - DNA, 31 bp, synthetic construct; identical to SEQ ID NO: 150
  source 1..31: mol_type = other DNA
  misc_feature 1: note = LNA
  misc_feature 12: note = LNA
  misc_feature 14: note = LNA
  misc_feature 31: note = LNA

SEQ ID NO: 152 - DNA, 31 bp, synthetic construct; identical to SEQ ID NO: 150
  source 1..31: mol_type = other DNA
  misc_feature 26..31: note = Phosphorothioate linkage
  misc_feature 1: note = LNA
  misc_feature 12: note = LNA
  misc_feature 14: note = LNA

SEQ ID NO: 153 - DNA, 31 bp, synthetic construct; identical to SEQ ID NO: 150
  misc_feature 26..29: note = Ribonucleotide
  source 1..31: mol_type = other DNA
  misc_feature 26..31: note = Phosphorothioate linkage
  misc_feature 1: note = LNA
  misc_feature 12: note = LNA
  misc_feature 14: note = LNA

SEQ ID NO: 154 - DNA, 31 bp, synthetic construct; identical to SEQ ID NO: 150
  source 1..31: mol_type = other DNA
  misc_feature 26..31: note = Phosphorothioate linkage
  misc_feature 1: note = LNA
  misc_feature 12: note = LNA
  misc_feature 14: note = LNA
  misc_feature 31: note = LNA

SEQ ID NO: 155 - DNA, 31 bp, synthetic construct; identical to SEQ ID NO: 150
  misc_feature 29..31: note = Ribonucleotide
  source 1..31: mol_type = other DNA
  misc_feature 1: note = LNA
  misc_feature 12: note = LNA
  misc_feature 14: note = LNA

SEQ ID NO: 156 - DNA, 31 bp, synthetic construct; identical to SEQ ID NO: 150
  misc_feature 29..31: note = Ribonucleotide
  source 1..31: mol_type = other DNA
  misc_feature 1: note = LNA
  misc_feature 12: note = LNA
  misc_feature 14: note = LNA
  misc_feature 31: note = LNA

SEQ ID NO: 157 - DNA, 28 bp, synthetic construct
  source 1..28: mol_type = other DNA
  misc_feature 1: note = LNA
  misc_feature 12: note = LNA
  misc_feature 14: note = LNA
gttcaaggacttggtccaggttgtatat

SEQ ID NO: 158 - DNA, 31 bp, synthetic construct
  source 1..31: mol_type = other DNA
  misc_feature 1: note = LNA
  misc_feature 12: note = LNA
  misc_feature 14: note = LNA
gttcaaggacttggtccaggttgtataatta

SEQ ID NO: 159 - DNA, 34 bp, synthetic construct
  source 1..34: mol_type = other DNA
  misc_feature 1: note = LNA
  misc_feature 12: note = LNA
  misc_feature 14: note = LNA
gttcaaggacttggtccaggttgtataattagtg

SEQ ID NO: 160 - DNA, 37 bp, synthetic construct
  source 1..37: mol_type = other DNA
  misc_feature 1: note = LNA
  misc_feature 12: note = LNA
  misc_feature 14: note = LNA
gttcaaggacttggtccaggttgtataattagtgagt

SEQ ID NO: 161 - DNA, 40 bp, synthetic construct
  source 1..40: mol_type = other DNA
  misc_feature 1: note = LNA
  misc_feature 12: note = LNA
  misc_feature 14: note = LNA
gttcaaggacttggtccaggttgtataattagtgagtgat

SEQ ID NO: 162 - DNA, 43 bp, synthetic construct
  source 1..43: mol_type = other DNA
  misc_feature 1: note = LNA
  misc_feature 12: note = LNA
  misc_feature 14: note = LNA
gttcaaggacttggtccaggttgtataattagtgagtgataac

SEQ ID NO: 163 - DNA, 28 bp, synthetic construct
  source 1..28: mol_type = other DNA
  misc_feature 23..28: note = Phosphorothioate linkage
  misc_feature 1: note = LNA
  misc_feature 12: note = LNA
  misc_feature 14: note = LNA
  misc_feature 28: note = LNA
gttcaaggacttggtccaggttgtatat

SEQ ID NO: 164 - DNA, 31 bp, synthetic construct; identical to SEQ ID NO: 158
  source 1..31: mol_type = other DNA
  misc_feature 26..31: note = Phosphorothioate linkage
  misc_feature 1: note = LNA
  misc_feature 12: note = LNA
  misc_feature 14: note = LNA

SEQ ID NO: 165 - DNA, 34 bp, synthetic construct; identical to SEQ ID NO: 159
  source 1..34: mol_type = other DNA
  misc_feature 29..34: note = Phosphorothioate linkage
  misc_feature 1: note = LNA
  misc_feature 12: note = LNA
  misc_feature 14: note = LNA

SEQ ID NO: 166 - DNA, 37 bp, synthetic construct; identical to SEQ ID NO: 160
  source 1..37: mol_type = other DNA
  misc_feature 32..37: note = Phosphorothioate linkage
  misc_feature 1: note = LNA
  misc_feature 12: note = LNA
  misc_feature 14: note = LNA

SEQ ID NO: 167 - DNA, 40 bp, synthetic construct; identical to SEQ ID NO: 161
  source 1..40: mol_type = other DNA
  misc_feature 35..40: note = Phosphorothioate linkage
  misc_feature 1: note = LNA
  misc_feature 12: note = LNA
  misc_feature 14: note = LNA

SEQ ID NO: 168 - DNA, 43 bp, synthetic construct; identical to SEQ ID NO: 162
  source 1..43: mol_type = other DNA
  misc_feature 38..43: note = Phosphorothioate linkage
  misc_feature 1: note = LNA
  misc_feature 12: note = LNA
  misc_feature 14: note = LNA

SEQ ID NO: 169 - DNA, 31 bp, synthetic construct
  source 1..31: mol_type = other DNA
  misc_feature 20..25: note = Phosphorothioate linkage
  misc_feature 1: note = LNA
  misc_feature 12: note = LNA
  misc_feature 14: note = LNA
gttcaaggacttggtccaggttgtatccggc

SEQ ID NO: 170 - DNA, 31 bp, synthetic construct; identical to SEQ ID NO: 169
  source 1..31: mol_type = other DNA
  misc_feature 20..25: note = Phosphorothioate linkage
  misc_feature 1: note = LNA
  misc_feature 12: note = LNA
  misc_feature 14: note = LNA

SEQ ID NO: 171 - DNA, 31 bp, synthetic construct; identical to SEQ ID NO: 169
  source 1..31: mol_type = other DNA
  misc_feature 20..25: note = Phosphorothioate linkage
  misc_feature 1: note = LNA
  misc_feature 12: note = LNA
  misc_feature 14: note = LNA

SEQ ID NO: 172 - DNA, 33 bp, synthetic construct
  source 1..33: mol_type = other DNA
  misc_feature 20..25: note = Phosphorothioate linkage
  misc_feature 1: note = LNA
  misc_feature 12: note = LNA
  misc_feature 14: note = LNA
gttcaaggacttggtccaggttgtataatgctg

SEQ ID NO: 173 - DNA, 33 bp, synthetic construct; identical to SEQ ID NO: 172
  source 1..33: mol_type = other DNA
  misc_feature 20..25: note = Phosphorothioate linkage
  misc_feature 1: note = LNA
  misc_feature 12: note = LNA
  misc_feature 14: note = LNA

SEQ ID NO: 174 - DNA, 31 bp, synthetic construct
  source 1..31: mol_type = other DNA
  misc_feature 20..25: note = Phosphorothioate linkage
  misc_feature 1: note = LNA
  misc_feature 12: note = LNA
  misc_feature 14: note = LNA
gttcaaggacttggtccaggttgtataaggc

SEQ ID NO: 175 - DNA, 31 bp, synthetic construct; identical to SEQ ID NO: 174
  source 1..31: mol_type = other DNA
  misc_feature 22..25: note = Phosphorothioate linkage
  misc_feature 1: note = LNA
  misc_feature 12: note = LNA
  misc_feature 14: note = LNA

SEQ ID NO: 176 - DNA, 31 bp, synthetic construct; identical to SEQ ID NO: 174
  source 1..31: mol_type = other DNA
  misc_feature 23..25: note = Phosphorothioate linkage
  misc_feature 1: note = LNA
  misc_feature 12: note = LNA
  misc_feature 14: note = LNA

SEQ ID NO: 177 - DNA, 31 bp, synthetic construct; identical to SEQ ID NO: 174
  source 1..31: mol_type = other DNA
  misc_feature 24..25: note = Phosphorothioate linkage
  misc_feature 1: note = LNA
  misc_feature 12: note = LNA
  misc_feature 14: note = LNA

SEQ ID NO: 178 - DNA, 32 bp, synthetic construct
  source 1..32: mol_type = other DNA
  misc_feature 20..25: note = Phosphorothioate linkage
  misc_feature 1: note = LNA
  misc_feature 12: note = LNA
  misc_feature 14: note = LNA
gttcaaggacttggtccaggttgtatgccggc

SEQ ID NO: 179 - DNA, 33 bp, synthetic construct
  source 1..33: mol_type = other DNA
  misc_feature 20..25: note = Phosphorothioate linkage
  misc_feature 1: note = LNA
  misc_feature 12: note = LNA
  misc_feature 14: note = LNA
gttcaaggacttggtccaggttgtattgccggc

SEQ ID NO: 180 - DNA, 34 bp, synthetic construct
  source 1..34: mol_type = other DNA
  misc_feature 20..25: note = Phosphorothioate linkage
  misc_feature 1: note = LNA
  misc_feature 12: note = LNA
  misc_feature 14: note = LNA
gttcaaggacttggtccaggttgtatttgccggc

SEQ ID NO: 181 - DNA, 32 bp, synthetic construct
  source 1..32: mol_type = other DNA
  misc_feature 20..25: note = Phosphorothioate linkage
  misc_feature 1: note = LNA
  misc_feature 12: note = LNA
  misc_feature 14: note = LNA
gttcaaggacttggtccaggttgtaagccggc

SEQ ID NO: 182 - DNA, 33 bp, synthetic construct
  source 1..33: mol_type = other DNA
  misc_feature 20..25: note = Phosphorothioate linkage
  misc_feature 1: note = LNA
  misc_feature 12: note = LNA
  misc_feature 14: note = LNA
gttcaaggacttggtccaggttgtaaagccggc

SEQ ID NO: 183 - DNA, 34 bp, synthetic construct
  source 1..34: mol_type = other DNA
  misc_feature 20..25: note = Phosphorothioate linkage
  misc_feature 1: note = LNA
  misc_feature 12: note = LNA
  misc_feature 14: note = LNA
gttcaaggacttggtccaggttgtaaaagccggc

SEQ ID NO: 184 - DNA, 31 bp, synthetic construct
  source 1..31: mol_type = other DNA
  misc_feature 26..31: note = Ribonucleotide
  misc_feature 31: note = 3' phosphate
  misc_feature 1: note = LNA
  misc_feature 12: note = LNA
  misc_feature 14: note = LNA
gttcaaggacttggtccaggttgtacgcgcg

SEQ ID NO: 185 - DNA, 31 bp, synthetic construct; identical to SEQ ID NO: 184
  misc_feature 26..31: note = Ribonucleotide
  source 1..31: mol_type = other DNA
  misc_feature 1: note = LNA
  misc_feature 12: note = LNA
  misc_feature 14: note = LNA
  misc_feature 31: note = LNA

SEQ ID NO: 186 - DNA, 31 bp, synthetic construct; identical to SEQ ID NO: 184
  misc_feature 26..31: note = Ribonucleotide
  source 1..31: mol_type = other DNA
  misc_feature 20..25: note = Phosphorothioate linkage
  misc_feature 1: note = LNA
  misc_feature 12: note = LNA
  misc_feature 14: note = LNA

SEQ ID NO: 187 - DNA, 49 bp, synthetic construct
  misc_feature 40..49: note = Ribonucleotide
  source 1..49: mol_type = other DNA
  misc_feature 1: note = LNA
  misc_feature 12: note = LNA
  misc_feature 14: note = LNA
gttcaaggacttggtccaggttgtataattagtgagacttcactaatta

SEQ ID NO: 188 - DNA, 49 bp, synthetic construct; identical to SEQ ID NO: 187
  misc_feature 36..49: note = Ribonucleotide
  source 1..49: mol_type = other DNA
  misc_feature 1: note = LNA
  misc_feature 12: note = LNA
  misc_feature 14: note = LNA

SEQ ID NO: 189 - DNA, 49 bp, synthetic construct; identical to SEQ ID NO: 187
  misc_feature 26..35: note = Ribonucleotide
  source 1..49: mol_type = other DNA
  misc_feature 1: note = LNA
  misc_feature 12: note = LNA
  misc_feature 14: note = LNA

SEQ ID NO: 190 - DNA, 49 bp, synthetic construct; identical to SEQ ID NO: 187
  misc_feature 26..39: note = Ribonucleotide
  source 1..49: mol_type = other DNA
  misc_feature 1: note = LNA
  misc_feature 12: note = LNA
  misc_feature 14: note = LNA

SEQ ID NO: 191 - DNA, 49 bp, synthetic construct; identical to SEQ ID NO: 187
  misc_feature 26..49: note = Ribonucleotide
  source 1..49: mol_type = other DNA
  misc_feature 1: note = LNA
  misc_feature 12: note = LNA
  misc_feature 14: note = LNA

SEQ ID NO: 192 - DNA, 55 bp, synthetic construct
  misc_feature 39..55: note = Ribonucleotide
  source 1..55: mol_type = other DNA
  misc_feature 1: note = LNA
  misc_feature 12: note = LNA
  misc_feature 14: note = LNA
gttcaaggacttggtccaggttgtataattagtgagtgctctcactcactaatta

SEQ ID NO: 193 - DNA, 43 bp, synthetic construct
  misc_feature 33..43: note = Ribonucleotide
  source 1..43: mol_type = other DNA
  misc_feature 1: note = LNA
  misc_feature 12: note = LNA
  misc_feature 14: note = LNA
gttcaaggacttggtccaggttgtataattagtgacctaatta

SEQ ID NO: 194 - DNA, 37 bp, synthetic construct
  misc_feature 30..37: note = Ribonucleotide
  source 1..37: mol_type = other DNA
gttcaaggacttggtccaggttgtataattagcatta

SEQ ID NO: 195 - DNA, 51 bp, synthetic construct
  misc_feature 36..41: note = Ribonucleotide
  source 1..51: mol_type = other DNA
  misc_feature 1: note = LNA
  misc_feature 12: note = LNA
  misc_feature 14: note = LNA
gttcaaggacttggtccaggttgtataattagtgagacacttcactaatta

SEQ ID NO: 196 - DNA, 49 bp, synthetic construct; identical to SEQ ID NO: 187
  misc_feature 36..49: note = Ribonucleotide
  source 1..49: mol_type = other DNA
  misc_feature 30..35: note = Phosphorothioate linkage
  misc_feature 1: note = LNA
  misc_feature 12: note = LNA
  misc_feature 14: note = LNA

SEQ ID NO: 197 - DNA, 51 bp, synthetic construct; identical to SEQ ID NO: 195
  misc_feature 36..51: note = Ribonucleotide
  source 1..51: mol_type = other DNA
  misc_feature 40..45: note = Phosphorothioate linkage
  misc_feature 1: note = LNA
  misc_feature 12: note = LNA
  misc_feature 14: note = LNA

SEQ ID NO: 198 - DNA, 51 bp, synthetic construct; identical to SEQ ID NO: 195
  misc_feature 36..51: note = Ribonucleotide
  source 1..51: mol_type = other DNA
  misc_feature 45..50: note = Phosphorothioate linkage
  misc_feature 1: note = LNA
  misc_feature 12: note = LNA
  misc_feature 14: note = LNA

SEQ ID NO: 199 - DNA, 51 bp, synthetic construct; identical to SEQ ID NO: 195
  misc_feature 36..51: note = Ribonucleotide
  source 1..51: mol_type = other DNA
  misc_feature 51: note = 3' phosphate
  misc_feature 1: note = LNA
  misc_feature 12: note = LNA
  misc_feature 14: note = LNA

SEQ ID NO: 200 - DNA, 49 bp, synthetic construct
  misc_feature 36..49: note = Ribonucleotide
  source 1..49: mol_type = other DNA
  misc_feature 1: note = LNA
  misc_feature 12: note = LNA
  misc_feature 14: note = LNA
gttcaaggacttggtccaggttgtataattagtgagatctcactaatta

SEQ ID NO: 201 - DNA, 49 bp, synthetic construct
  misc_feature 36..49: note = Ribonucleotide
  source 1..49: mol_type = other DNA
  misc_feature 1: note = LNA
  misc_feature 12: note = LNA
  misc_feature 14: note = LNA
gttcaaggacttggtccaggttgtataattagtgagacctcactaatta

SEQ ID NO: 202 - DNA, 25 bp, synthetic construct
  source 1..25: mol_type = other DNA
  misc_feature 24..25: note = Phosphorothioate linkage
  misc_feature 1: note = LNA
  misc_feature 13: note = LNA
  misc_feature 25: note = LNA
gttcaaggacttggtccaggttgta

SEQ ID NO: 203 - DNA, 25 bp, synthetic construct
  source 1..25: mol_type = other DNA
  misc_feature 20..25: note = Phosphorothioate linkage
  misc_feature 1: note = LNA
  misc_feature 13: note = LNA
gttcaaggacttggtccaggttgta

SEQ ID NO: 204 - DNA, 25 bp, synthetic construct
  source 1..25: mol_type = other DNA
  misc_feature 20..25: note = Phosphorothioate linkage
  misc_feature 25: note = 3' phosphate
  misc_feature 1: note = LNA
  misc_feature 13: note = LNA
gttcaaggacttggtccaggttgta

SEQ ID NO: 205 - DNA, 25 bp, synthetic construct
  source 1..25: mol_type = other DNA
  misc_feature 18..25: note = Phosphorothioate linkage
  misc_feature 25: note = 3' phosphate
  misc_feature 1: note = LNA
  misc_feature 13: note = LNA
gttcaaggacttggtccaggttgta

SEQ ID NO: 206 - DNA, 38 bp, synthetic construct; identical to SEQ ID NO: 51
  source 1..38: mol_type = other DNA
  misc_feature 1..6: note = Phosphorothioate linkage
  misc_feature 25: note = LNA
  misc_feature 27: note = LNA

SEQ ID NO: 207 - DNA, 38 bp, synthetic construct; identical to SEQ ID NO: 51
  source 1..38: mol_type = other DNA
  misc_feature 1..6: note = Phosphorothioate linkage
  misc_feature 14: note = LNA
  misc_feature 25: note = LNA
  misc_feature 27: note = LNA

SEQ ID NO: 208 - DNA, 31 bp, synthetic construct
  misc_feature 1..6: note = Ribonucleotide
  source 1..31: mol_type = other DNA
  misc_feature 7: note = LNA
  misc_feature 18: note = LNA
  misc_feature 20: note = LNA
cgcgcggttcaaggacttggtccaggttgta

SEQ ID NO: 209 - DNA, 31 bp, synthetic construct
  source 1..31: mol_type = other DNA
  misc_feature 7: note = LNA
  misc_feature 18: note = LNA
  misc_feature 20: note = LNA
ccccccgttcaaggacttggtccaggttgta

SEQ ID NO: 210 - DNA, 33 bp, synthetic construct
  misc_feature 1..8: note = Ribonucleotide
  source 1..33: mol_type = other DNA
  misc_feature 9: note = LNA
  misc_feature 20: note = LNA
  misc_feature 22: note = LNA
cgcgcgcggttcaaggacttggtccaggttgta

SEQ ID NO: 211 - DNA, 35 bp, synthetic construct
  misc_feature 1..10: note = Ribonucleotide
  source 1..35: mol_type = other DNA
  misc_feature 11: note = LNA
  misc_feature 22: note = LNA
  misc_feature 24: note = LNA
cgcgcgcgcggttcaaggacttggtccaggttgta

SEQ ID NO: 212 - DNA, 31 bp, synthetic construct
  misc_feature 1..6: note = Ribonucleotide
  source 1..31: mol_type = other DNA
  misc_feature 7: note = LNA
  misc_feature 20: note = LNA
  misc_feature 22: note = LNA
gcgcgcgttcaaggacttggtccaggttgta

SEQ ID NO: 213 - DNA, 31 bp, synthetic construct
  misc_feature 1..6: note = Ribonucleotide
  source 1..31: mol_type = other DNA
  misc_feature 7: note = LNA
  misc_feature 20: note = LNA
  misc_feature 22: note = LNA
cccggggttcaaggacttggtccaggttgta

SEQ ID NO: 214 - DNA, 27 bp, synthetic construct
  source 1..27: mol_type = other DNA
  misc_feature 1: note = LNA
  misc_feature 14: note = LNA
  misc_feature 16: note = LNA
ctgttcaaggacttggtccaggttgta

SEQ ID NO: 215 - DNA, 27 bp, synthetic construct
  source 1..27: mol_type = other DNA
  misc_feature 2: note = LNA
  misc_feature 14: note = LNA
  misc_feature 16: note = LNA
ctgttcaaggacttggtccaggttgta

SEQ ID NO: 216 - DNA, 28 bp, synthetic construct
  source 1..28: mol_type = other DNA
  misc_feature 1: note = LNA
  misc_feature 15: note = LNA
  misc_feature 17: note = LNA
cctgttcaaggacttggtccaggttgta

SEQ ID NO: 217 - DNA, 28 bp, synthetic construct
  source 1..28: mol_type = other DNA
  misc_feature 2: note = LNA
  misc_feature 15: note = LNA
  misc_feature 17: note = LNA
cctgttcaaggacttggtccaggttgta

SEQ ID NO: 218 - DNA, 28 bp, synthetic construct
  source 1..28: mol_type = other DNA
  misc_feature 3: note = LNA
  misc_feature 15: note = LNA
  misc_feature 17: note = LNA
cctgttcaaggacttggtccaggttgta

SEQ ID NO: 219 - DNA, 25 bp, synthetic construct
  source 1..25: mol_type = other DNA
  misc_feature 1: note = adapter-linked
  misc_feature 1: note = LNA
  misc_feature 12: note = LNA
  misc_feature 14: note = LNA
gttcaaggacttggtccaggttgta

SEQ ID NO: 220 - DNA, 25 bp, synthetic construct
  source 1..25: mol_type = other DNA
  misc_feature 1: note = LNA
  misc_feature 12: note = LNA
  misc_feature 14: note = LNA
  misc_feature 1: note = adapter-linked
gttcaaggacttggtccaggttgta

SEQ ID NO: 221 - DNA, 25 bp, synthetic construct
  source 1..25: mol_type = other DNA
  misc_feature 1: note = Phosphorothioate linkage
  misc_feature 1: note = LNA
  misc_feature 12: note = LNA
  misc_feature 14: note = LNA
  misc_feature 1: note = adapter-linked
gttcaaggacttggtccaggttgta

SEQ ID NO: 222 - DNA, 25 bp, synthetic construct
  source 1..25: mol_type = other DNA
  misc_feature 25: note = adapter-linked
  misc_feature 1: note = LNA
  misc_feature 12: note = LNA
  misc_feature 14: note = LNA
gttcaaggacttggtccaggttgta

SEQ ID NO: 223 - DNA, 25 bp, synthetic construct
  source 1..25: mol_type = other DNA
  misc_feature 25: note = adapter-linked
  misc_feature 1: note = LNA
  misc_feature 12: note = LNA
  misc_feature 14: note = LNA
gttcaaggacttggtccaggttgta

SEQ ID NO: 224 - DNA, 25 bp, synthetic construct
  source 1..25: mol_type = other DNA
  misc_feature 1: note = LNA
  misc_feature 12: note = LNA
  misc_feature 14: note = LNA
  misc_feature 25: note = adapter-linked
gttcaaggacttggtccaggttgta

SEQ ID NO: 225 - DNA, 25 bp, synthetic construct
  source 1..25: mol_type = other DNA
  misc_feature 20..25: note = Phosphorothioate linkage
  misc_feature 25: note = adapter-linked
  misc_feature 1: note = LNA
  misc_feature 12: note = LNA
  misc_feature 14: note = LNA
gttcaaggacttggtccaggttgta

SEQ ID NO: 226 - DNA, 25 bp, synthetic construct
  source 1..25: mol_type = other DNA
  misc_feature 1: note = LNA
  misc_feature 12: note = LNA
  misc_feature 14: note = LNA
  misc_feature 25: note = adapter-linked
gttcaaggacttggtccaggttgta

SEQ ID NO: 227 - DNA, 25 bp, synthetic construct
  source 1..25: mol_type = other DNA
  misc_feature 1: note = LNA
  misc_feature 12: note = LNA
  misc_feature 14: note = LNA
  misc_feature 25: note = adapter-linked
gttcaaggacttggtccaggttgta

SEQ ID NO: 228 - DNA, 25 bp, synthetic construct
  source 1..25: mol_type = other DNA
  misc_feature 1: note = LNA
  misc_feature 12: note = LNA
  misc_feature 14: note = LNA
  misc_feature 25: note = adapter-linked
gttcaaggacttggtccaggttgta

SEQ ID NO: 229 - DNA, 25 bp, synthetic construct
  source 1..25: mol_type = other DNA
  misc_feature 1: note = LNA
  misc_feature 12: note = LNA
  misc_feature 14: note = LNA
  misc_feature 25: note = adapter-linked
gttcaaggacttggtccaggttgta

SEQ ID NO: 230 - DNA, 25 bp, synthetic construct
  source 1..25: mol_type = other DNA
  misc_feature 1..2: note = Phosphorothioate linkage
  misc_feature 3..4: note = Phosphorothioate linkage
  misc_feature 1: note = LNA
  misc_feature 12: note = LNA
  misc_feature 14: note = LNA
gttcaaggacttggtccaggttgta

SEQ ID NO: 231 - DNA, 25 bp, synthetic construct
  source 1..25: mol_type = other DNA
  misc_feature 1..2: note = Phosphorothioate linkage
  misc_feature 3..4: note = Phosphorothioate linkage
  misc_feature 5..6: note = Phosphorothioate linkage
  misc_feature 1: note = LNA
  misc_feature 12: note = LNA
  misc_feature 14: note = LNA
gttcaaggacttggtccaggttgta

SEQ ID NO: 232 - DNA, 25 bp, synthetic construct
  source 1..25: mol_type = other DNA
  misc_feature 8..10: note = Phosphorothioate linkage
  misc_feature 1: note = LNA
  misc_feature 12: note = LNA
  misc_feature 14: note = LNA
gttcaaggacttggtccaggttgta

SEQ ID NO: 233 - DNA, 25 bp, synthetic construct
  source 1..25: mol_type = other DNA
  misc_feature 6..8: note = Phosphorothioate linkage
  misc_feature 1: note = LNA
  misc_feature 12: note = LNA
  misc_feature 14: note = LNA
gttcaaggacttggtccaggttgta

SEQ ID NO: 234 - DNA, 25 bp, synthetic construct
  source 1..25: mol_type = other DNA
  misc_feature 4..6: note = Phosphorothioate linkage
  misc_feature 1: note = LNA
  misc_feature 12: note = LNA
  misc_feature 14: note = LNA
gttcaaggacttggtccaggttgta

SEQ ID NO: 235 - DNA, 25 bp, synthetic construct
  source 1..25: mol_type = other DNA
  misc_feature 15..19: note = Phosphorothioate linkage
  misc_feature 1: note = LNA
  misc_feature 12: note = LNA
  misc_feature 14: note = LNA
gttcaaggacttggtccaggttgta

SEQ ID NO: 236 - DNA, 25 bp, synthetic construct
  source 1..25: mol_type = other DNA
  misc_feature 22..23: note = Phosphorothioate linkage
  misc_feature 24..25: note = Phosphorothioate linkage
  misc_feature 1: note = LNA
  misc_feature 12: note = LNA
  misc_feature 14: note = LNA
gttcaaggacttggtccaggttgta

SEQ ID NO: 237 - DNA, 25 bp, synthetic construct
  source 1..25: mol_type = other DNA
  misc_feature 20..21: note = Phosphorothioate linkage
  misc_feature 22..23: note = Phosphorothioate linkage
  misc_feature 24..25: note = Phosphorothioate linkage
  misc_feature 1: note = LNA
  misc_feature 12: note = LNA
  misc_feature 14: note = LNA
gttcaaggacttggtccaggttgta

SEQ ID NO: 238 - DNA, 25 bp, synthetic construct
  source 1..25: mol_type = other DNA
  misc_feature 15..17: note = Phosphorothioate linkage
  misc_feature 1: note = LNA
  misc_feature 12: note = LNA
  misc_feature 14: note = LNA
gttcaaggacttggtccaggttgta

SEQ ID NO: 239 - DNA, 25 bp, synthetic construct
  source 1..25: mol_type = other DNA
  misc_feature 17..19: note = Phosphorothioate linkage
  misc_feature 1: note = LNA
  misc_feature 12: note = LNA
  misc_feature 14: note = LNA
gttcaaggacttggtccaggttgta

SEQ ID NO: 240 - DNA, 25 bp, synthetic construct
  source 1..25: mol_type = other DNA
  misc_feature 19..21: note = Phosphorothioate linkage
  misc_feature 1: note = LNA
  misc_feature 12: note = LNA
  misc_feature 14: note = LNA
gttcaaggacttggtccaggttgta